European Patent Specification EP 4 294 424 B1, published February 11, 2026. Title: Composition. Applicant: Zealand Pharma A/S. Application EP22707673.4. The sequence listing filed with the application follows.

SEQUENCE LISTING (178 sequences)

SEQ ID NO: 1 - protein, 33 aa, Artificial Sequence
  GLP-1/GLP-1 dual agonist peptide
  MISC_FEATURE (2)..(2): Xaa is Aib or G
  MISC_FEATURE (5)..(5): Xaa is T or S with at least one of Xaa at position 5 or 7 being a T
  MISC_FEATURE (7)..(7): Xaa is T or S with at least one of Xaa at position 5 or 7 being a T
  MISC_FEATURE (8)..(8): Xaa is S, E or D
  MISC_FEATURE (10)..(10): Xaa is L, M, V or a residue of K, k (D-lys), R, Orn, Dap or Dab in which the side chain is conjugated to a substituent
  MISC_FEATURE (11)..(11): Xaa is A, N or S
  MISC_FEATURE (15)..(15): Xaa is D or E
  MISC_FEATURE (16)..(16): Xaa is G, E, A or a residue of K, k (D-lys), R, Orn, Dap or Dab in which the side chain is conjugated to a substituent
  MISC_FEATURE (17)..(17): Xaa is Q, E, K, L or a residue of K, k (D-lys), R, Orn, Dap or Dab in which the side chain is conjugated to a substituent
  MISC_FEATURE (19)..(19): Xaa is A, V or S
  MISC_FEATURE (20)..(20): Xaa is R, K or a residue of K, k (D-lys), R, Orn, Dap or Dab in which the side chain is conjugated to a substituent
  MISC_FEATURE (21)..(21): Xaa is D, L or E
  MISC_FEATURE (24)..(24): Xaa is A, N or  S
  MISC_FEATURE (27)..(27): Xaa is I, Q, K, H or Y
  MISC_FEATURE (28)..(28): Xaa is Q, E, A, H, Y, L, K, R or S
  MISC_FEATURE (29)..(29): Xaa is H, Y, K or Q
  MISC_FEATURE (33)..(33): Xaa is D or  E
HXEGXFXXEXXTILXXXAXXXFIXWLXXXKITX

SEQ ID NO: 2 - protein, 33 aa, Artificial Sequence
  GLP-1/GLP-2 Dual agonist peptide
  MISC_FEATURE (2)..(2): Xaa is Aib or G
  MISC_FEATURE (5)..(5): Xaa is T or S
  MISC_FEATURE (7)..(7): Xaa is T or S
  MISC_FEATURE (16)..(16): Xaa is G or a residue of K, k (D-lys), R, Orn, Dap or Dab in which the side chain is conjugated to a substituent
  MISC_FEATURE (17)..(17): Xaa is Q, E, K, L or a residue of K, k (D-lys), R, Orn, Dap or Dab in which the side chain is conjugated to a substituent
  MISC_FEATURE (21)..(21): Xaa is D or L
  MISC_FEATURE (28)..(28): Xaa is Q, E, A, H, Y, L, K, R or S
  MISC_FEATURE (29)..(29): Xaa is H, Y or Q
HXEGXFXSELATILDXXAARXFIAWLIXXKITD

SEQ ID NO: 3 - protein, 33 aa, Artificial Sequence
  GLP-1/GLP-2 dual agonist peptide
  MOD_RES (2)..(2): Aib
  MISC_FEATURE (5)..(5): Xaa is T or S with at least one of Xaa at position 5 or 7 being a T
  MISC_FEATURE (7)..(7): Xaa is T or S with at least one of Xaa at position 5 or 7 being a T
  MISC_FEATURE (10)..(10): Xaa is L or a residue of K, k (D-lys), R, Orn, Dap or Dab in which the side chain is conjugated to a substituent
  MISC_FEATURE (16)..(16): Xaa is G, E, A or a residue of K, k (D-lys), R, Orn, Dap or Dab in which the side chain is conjugated to a substituent
  MISC_FEATURE (17)..(17): Xaa is Q, E, K, L or a residue of K, k (D-lys), R, Orn, Dap or Dab in which the side chain is conjugated to a substituent
  MISC_FEATURE (20)..(20): Xaa is R or a residue of K, k (D-lys), R, Orn, Dap or Dab in which the side chain is conjugated to a substituent
  MISC_FEATURE (21)..(21): Xaa is D or L
  MISC_FEATURE (28)..(28): Xaa is E, A or Q
  MISC_FEATURE (29)..(29): Xaa is H, Y or Q
HXEGXFXSEXATILDXXAAXXFIAWLIXXKITD

SEQ ID NO: 4 - protein, 33 aa, Artificial Sequence; identical to SEQ ID NO: 2
  GLP-1/GLP-2 Dual agonist peptide
  MOD_RES (2)..(2): Aib
  MISC_FEATURE (5)..(5): Xaa is T or S with at least one of Xaa at position 5 or 7 being a T
  MISC_FEATURE (7)..(7): Xaa is T or S with at least one of Xaa at position 5 or 7 being a T
  MISC_FEATURE (16)..(16): Xaa is G or a residue of K, k (D-lys), R, Orn, Dap or Dab in which the side chain is conjugated to a substituent
  MISC_FEATURE (17)..(17): Xaa is E, K, L or a residue of K, k (D-lys), R, Orn, Dap or Dab in which the side chain is conjugated to a substituent
  MISC_FEATURE (21)..(21): Xaa is D or L
  MISC_FEATURE (28)..(28): Xaa is E or A
  MISC_FEATURE (29)..(29): Xaa is H, Y or Q

SEQ ID NO: 5 - protein, 33 aa, Artificial Sequence
  GLP-1/GLP-2 Dual agonist peptide
  MOD_RES (2)..(2): Aib
  MISC_FEATURE (5)..(5): Xaa is T or S where at least one of Xaa at position 5 or 7 is a T
  MISC_FEATURE (7)..(7): Xaa is T or S where at least one of Xaa at position 5 or 7 is a T
  MISC_FEATURE (16)..(16): Xaa is a residue of K, k (D-lys), R, Orn, Dap or Dab in which the side chain is conjugated to a substituent
  MISC_FEATURE (28)..(28): Xaa is Q, E, A, H, Y, L, K, R or S, e.g. Q, E, A, H, Y or L
  MISC_FEATURE (29)..(29): Xaa is H, Y or Q
HXEGXFXSELATILDXQAARDFIAWLIXXKITD

SEQ ID NO: 6 - protein, 6 aa, Artificial Sequence
  GLP-1/GLP-2 Dual agonist peptide
  PEPTIDE (1)..(6): Xaa is D-lys
  MISC_FEATURE (1)..(6)
XXXXXX

SEQ ID NO: 7 - protein, 6 aa, Artificial Sequence
  GLP-1/GLP-2 Dual agonist peptide
EKEKEK

SEQ ID NO: 8 - protein, 6 aa, Artificial Sequence
  GLP-1/GLP-2 Dual agonist peptide
  MISC_FEATURE (2)..(2): Xaa is D-lys
  MISC_FEATURE (4)..(4): Xaa is D-lys
  MISC_FEATURE (6)..(6): Xaa is D-lys
EXEXEX

SEQ ID NO: 9 - protein, 6 aa, Artificial Sequence
  GLP-1/GLP-2 Dual agonist peptide
AKAAEK

SEQ ID NO: 10 - protein, 6 aa, Artificial Sequence
  GLP-1/GLP-2 Dual agonist peptide
AKEKEK

SEQ ID NO: 11 - protein, 6 aa, Artificial Sequence
  GLP-1/GLP-2 Dual agonist peptide
ATILEK

SEQ ID NO: 12 - protein, 6 aa, Artificial Sequence
  GLP-1/GLP-2 Dual agonist peptide
  MISC_FEATURE (6)..(6): Xaa is a residue of K, k (D-lys), R, Orn, Dap or Dab in which the side chain is conjugated to a substituent
EKEKEX

SEQ ID NO: 13 - protein, 6 aa, Artificial Sequence
  GLP-1/GLP-2 Dual agonist peptide
  MISC_FEATURE (2)..(2): Xaa is D-lys
  MISC_FEATURE (4)..(4): Xaa is D-lys
  MISC_FEATURE (6)..(6): Xaa is a residue of K, k (D-lys), R, Orn, Dap or Dab in which the side chain is conjugated to a substituent
EXEXEX

SEQ ID NO: 14 - protein, 6 aa, Artificial Sequence
  GLP-1/GLP-2 Dual agonist peptide
  MISC_FEATURE (6)..(6): Xaa is a residue of K, k (D-lys), R, Orn, Dap or Dab in which the side chain is conjugated to a substituent
AKAAEX

SEQ ID NO: 15 - protein, 6 aa, Artificial Sequence
  GLP-1/GLP-2 Dual agonist peptide
  MISC_FEATURE (6)..(6): Xaa is a residue of K, k (D-lys), R, Orn, Dap or Dab in which the side chain is conjugated to a substituent
AKEKEX

SEQ ID NO: 16 - protein, 6 aa, Artificial Sequence
  GLP-1/GLP-2 Dual agonist peptide
  MISC_FEATURE (6)..(6): xaa is a residue of K, k (D-lys), R, Orn, Dap or Dab in which the side chain is conjugated to a substituent
ATILEX

SEQ ID NO: 17 - protein, 33 aa, Artificial Sequence
  GLP-1/GLP-2 Dual agonist peptide
  MOD_RES (2)..(2): Aib
  MISC_FEATURE (16)..(16): Xaa is a residue of K, k (D-lys), R, Orn, Dap or Dab in which the side chain is conjugated to a substituent
HXEGTFSSELATILDXEAARDFIAWLIEHKITD

SEQ ID NO: 18 - protein, 33 aa, Artificial Sequence
  GLP-1/GLP-2 Dual agonist peptide
  MOD_RES (2)..(2): Aib
  MISC_FEATURE (16)..(16): Xaa is a residue of K, k (D-lys), R, Orn, Dap or Dab in which the side chain is conjugated to a substituent
HXEGSFTSELATILDXEAARDFIAWLIEHKITD

SEQ ID NO: 19 - protein, 33 aa, Artificial Sequence
  GLP-1/GLP-2 Dual agonist peptide
  MOD_RES (2)..(2): Aib
  MISC_FEATURE (16)..(16): Xaa is a residue of K, k (D-lys), R, Orn, Dap or Dab in which the side chain is conjugated to a substituent
HXEGTFTSELATILDXEAARDFIAWLIEHKITD

SEQ ID NO: 20 - protein, 33 aa, Artificial Sequence
  GLP-1/GLP-2 Dual agonist peptide
  MOD_RES (2)..(2): Aib
  MISC_FEATURE (16)..(16): Xaa is a residue of K, k (D-lys), R, Orn, Dap or Dab in which the side chain is conjugated to a substituent
HXEGTFSSELATILDXKAARDFIAWLIEHKITD

SEQ ID NO: 21 - protein, 33 aa, Artificial Sequence
  GLP-1/GLP-2 Dual agonist peptide
  MOD_RES (2)..(2): Aib
  MISC_FEATURE (16)..(16): Xaa is a residue of K, k (D-lys), R, Orn, Dap or Dab in which the side chain is conjugated to a substituent
HXEGSFTSELATILDXKAARDFIAWLIEHKITD

SEQ ID NO: 22 - protein, 33 aa, Artificial Sequence
  GLP-1/GLP-2 Dual agonist peptide
  MOD_RES (2)..(2): Aib
  MISC_FEATURE (16)..(16): Xaa is a residue of K, k (D-lys), R, Orn, Dap or Dab in which the side chain is conjugated to a substituent
HXEGTFTSELATILDXKAARDFIAWLIEHKITD

SEQ ID NO: 23 - protein, 33 aa, Artificial Sequence
  GLP-1/GLP-2 Dual agonist peptide
  MOD_RES (2)..(2): Aib
  MISC_FEATURE (17)..(17): Xaa is a residue of K, k (D-lys), R, Orn, Dap or Dab in which the side chain is conjugated to a substituent
HXEGTFSSELATILDGXAARDFIAWLIEHKITD

SEQ ID NO: 24 - protein, 33 aa, Artificial Sequence
  GLP-1/GLP-2 Dual agonist peptide
  MOD_RES (2)..(2): Aib
  MISC_FEATURE (17)..(17): Xaa is a residue of K, k (D-lys), R, Orn, Dap or Dab in which the side chain is conjugated to a substituent
HXEGSFTSELATILDGXAARDFIAWLIEHKITD

SEQ ID NO: 25 - protein, 33 aa, Artificial Sequence
  GLP-1/GLP-2 Dual agonist peptide
  MOD_RES (2)..(2): Aib
  MISC_FEATURE (17)..(17): Xaa is a residue of K, k (D-lys), R, Orn, Dap or Dab in which the side chain is conjugated to a substituent
HXEGTFTSELATILDGXAARDFIAWLIEHKITD

SEQ ID NO: 26 - protein, 33 aa, Artificial Sequence
  GLP-1/GLP-2 Dual agonist peptide
  MOD_RES (2)..(2): Aib
  MISC_FEATURE (16)..(16): Xaa is a residue of K, k (D-lys), R, Orn, Dap or Dab in which the side chain is conjugated to a substituent
HXEGTFSSELATILDXLAARDFIAWLIEHKITD

SEQ ID NO: 27 - protein, 33 aa, Artificial Sequence
  GLP-1/GLP-2 Dual agonist peptide
  MOD_RES (2)..(2): Aib
  MISC_FEATURE (16)..(16): Xaa is a residue of K, k (D-lys), R, Orn, Dap or Dab in which the side chain is conjugated to a substituent
HXEGSFTSELATILDXLAARDFIAWLIEHKITD

SEQ ID NO: 28 - protein, 33 aa, Artificial Sequence
  GLP-1/GLP-2 Dual agonist peptide
  MOD_RES (2)..(2): Aib
  MISC_FEATURE (16)..(16): Xaa is a residue of K, k (D-lys), R, Orn, Dap or Dab in which the side chain is conjugated to a substituent
HXEGTFTSELATILDXLAARDFIAWLIEHKITD

SEQ ID NO: 29 - protein, 33 aa, Artificial Sequence
  GLP-1/GLP-2 Dual agonist peptide
  MOD_RES (2)..(2): Aib
  MISC_FEATURE (16)..(16): Xaa is a residue of K, k (D-lys), R, Orn, Dap or Dab in which the side chain is conjugated to a substituent
HXEGTFSSELATILDXLAARDFIAWLIAHKITD

SEQ ID NO: 30 - protein, 33 aa, Artificial Sequence
  GLP-1/GLP-2 Dual agonist peptide
  MOD_RES (2)..(2): Aib
  MISC_FEATURE (16)..(16): Xaa is a residue of K, k (D-lys), R, Orn, Dap or Dab in which the side chain is conjugated to a substituent
HXEGSFTSELATILDXLAARDFIAWLIAHKITD

SEQ ID NO: 31 - protein, 33 aa, Artificial Sequence
  GLP-1/GLP-2 Dual agonist peptide
  MOD_RES (2)..(2): Aib
  MISC_FEATURE (16)..(16): Xaa is a residue of K, k (D-lys), R, Orn, Dap or Dab in which the side chain is conjugated to a substituent
HXEGTFTSELATILDXLAARDFIAWLIAHKITD

SEQ ID NO: 32 - protein, 33 aa, Artificial Sequence
  GLP-1/GLP-2 Dual agonist peptide
  MOD_RES (2)..(2): Aib
  MISC_FEATURE (16)..(16): Xaa is a residue of K, k (D-lys), R, Orn, Dap or Dab in which the side chain is conjugated to a substituent
HXEGTFTSELATILDXEAARLFIAWLIEHKITD

SEQ ID NO: 33 - protein, 33 aa, Artificial Sequence
  GLP-1/GLP-2 Dual agonist peptide
  MOD_RES (2)..(2): Aib
  MISC_FEATURE (16)..(16): Xaa is a residue of K, k (D-lys), R, Orn, Dap or Dab in which the side chain is conjugated to a substituent
HXEGTFSSELATILDXQAARDFIAWLIQHKITD

SEQ ID NO: 34 - protein, 33 aa, Artificial Sequence
  GLP-1/GLP-2 Dual agonist peptide
  MOD_RES (2)..(2): Aib
  MISC_FEATURE (16)..(16): Xaa is a residue of K, k (D-lys), R, Orn, Dap or Dab in which the side chain is conjugated to a substituent
HXEGSFTSELATILDXQAARDFIAWLIQHKITD

SEQ ID NO: 35 - protein, 33 aa, Artificial Sequence
  GLP-1/GLP-2 Dual agonist peptide
  MOD_RES (2)..(2): Aib
  MISC_FEATURE (16)..(16): Xaa is a residue of K, k (D-lys), R, Orn, Dap or Dab in which the side chain is conjugated to a substituent
HXEGTFTSELATILDXQAARDFIAWLIQHKITD

SEQ ID NO: 36 - protein, 33 aa, Artificial Sequence
  GLP-1/GLP-2 Dual agonist peptide
  MOD_RES (2)..(2): Aib
  MISC_FEATURE (16)..(16): Xaa is a residue of K, k (D-lys), R, Orn, Dap or Dab in which the side chain is conjugated to a substituent
HXEGTFSSELATILDXQAARDFIAWLIEHKITD

SEQ ID NO: 37 - protein, 33 aa, Artificial Sequence
  GLP-1/GLP-2 Dual agonist peptide
  MOD_RES (2)..(2): Aib
  MISC_FEATURE (16)..(16): Xaa is a residue of K, k (D-lys), R, Orn, Dap or Dab in which the side chain is conjugated to a substituent
HXEGTFSSELATILDXQAARDFIAWLIAHKITD

SEQ ID NO: 38 - protein, 33 aa, Artificial Sequence
  GLP-1/GLP-2 Dual agonist peptide
  MOD_RES (2)..(2): Aib
  MISC_FEATURE (16)..(16): Xaa is a residue of K, k (D-lys), R, Orn, Dap or Dab in which the side chain is conjugated to a substituent
HXEGSFTSELATILDXQAARDFIAWLIAHKITD

SEQ ID NO: 39 - protein, 33 aa, Artificial Sequence
  GLP-1/GLP-2 Dual agonist peptide
  MOD_RES (2)..(2): Aib
  MISC_FEATURE (16)..(16): Xaa is a residue of K, k (D-lys), R, Orn, Dap or Dab in which the side chain is conjugated to a substituent
HXEGTFTSELATILDXQAARDFIAWLIAHKITD

SEQ ID NO: 40 - protein, 33 aa, Artificial Sequence
  GLP-1/GLP-2 Dual agonist peptide
  MOD_RES (2)..(2): Aib
  MISC_FEATURE (16)..(16): Xaa is a residue of K, k (D-lys), R, Orn, Dap or Dab in which the side chain is conjugated to a substituent
HXEGSFTSELATILDXQAARDFIAWLIEHKITD

SEQ ID NO: 41 - protein, 33 aa, Artificial Sequence
  GLP-1/GLP-2 Dual agonist peptide
  MOD_RES (2)..(2): Aib
  MISC_FEATURE (16)..(16): Xaa is a residue of K, k (D-lys), R, Orn, Dap or Dab in which the side chain is conjugated to a substituent
HXEGTFTSELATILDXQAARDFIAWLIEHKITD

SEQ ID NO: 42 - protein, 33 aa, Artificial Sequence
  GLP-1/GLP-2 Dual agonist peptide
  MOD_RES (2)..(2): Aib
  MISC_FEATURE (16)..(16): Xaa is a residue of K, k (D-lys), R, Orn, Dap or Dab in which the side chain is conjugated to a substituent
HXEGSFTSELATILDXQAARDFIAWLIHHKITD

SEQ ID NO: 43 - protein, 33 aa, Artificial Sequence
  GLP-1/GLP-2 Dual agonist peptide
  MOD_RES (2)..(2): Aib
  MISC_FEATURE (16)..(16): Xaa is a residue of K, k (D-lys), R, Orn, Dap or Dab in which the side chain is conjugated to a substituent
HXEGSFTSELATILDXQAARDFIAWLIYHKITD

SEQ ID NO: 44 - protein, 33 aa, Artificial Sequence
  GLP-1/GLP-2 Dual agonist peptide
  MOD_RES (2)..(2): Aib
  MISC_FEATURE (16)..(16): Xaa is a residue of K, k (D-lys), R, Orn, Dap or Dab in which the side chain is conjugated to a substituent
HXEGSFTSELATILDXQAARDFIAWLILHKITD

SEQ ID NO: 45 - protein, 33 aa, Artificial Sequence
  GLP-1/GLP-2 Dual agonist peptide
  MOD_RES (2)..(2): Aib
  MISC_FEATURE (16)..(16): Xaa is a residue of K, k (D-lys), R, Orn, Dap or Dab in which the side chain is conjugated to a substituent
HXEGSFTSELATILDXQAARDFIAWLIKHKITD

SEQ ID NO: 46 - protein, 33 aa, Artificial Sequence
  GLP-1/GLP-2 Dual agonist peptide
  MOD_RES (2)..(2): Aib
  MISC_FEATURE (16)..(16): Xaa is a residue of K, k (D-lys), R, Orn, Dap or Dab in which the side chain is conjugated to a substituent
HXEGSFTSELATILDXQAARDFIAWLIRHKITD

SEQ ID NO: 47 - protein, 33 aa, Artificial Sequence
  GLP-1/GLP-2 Dual agonist peptide
  MOD_RES (2)..(2): Aib
  MISC_FEATURE (16)..(16): Xaa is a residue of K, k (D-lys), R, Orn, Dap or Dab in which the side chain is conjugated to a substituent
HXEGSFTSELATILDXQAARDFIAWLISHKITD

SEQ ID NO: 48 - protein, 33 aa, Artificial Sequence
  GLP-1/GLP-2 Dual agonist peptide
  MOD_RES (2)..(2): Aib
  MISC_FEATURE (16)..(16): Xaa is a residue of K, k (D-lys), R, Orn, Dap or Dab in which the side chain is conjugated to a substituent
HXEGSFTSELATILDXQAARDFIAWLQQHKITD

SEQ ID NO: 49 - protein, 33 aa, Artificial Sequence
  GLP-1/GLP-2 Dual agonist peptide
  MOD_RES (2)..(2): Aib
  MISC_FEATURE (16)..(16): Xaa is a residue of K, k (D-lys), R, Orn, Dap or Dab in which the side chain is conjugated to a substituent
HXEGSFTSELATILDXQAARDFIAWLYQHKITD

SEQ ID NO: 50 - protein, 33 aa, Artificial Sequence
  GLP-1/GLP-2 Dual agonist peptide
  MOD_RES (2)..(2): Aib
  MISC_FEATURE (16)..(16): Xaa is a residue of K, k (D-lys), R, Orn, Dap or Dab in which the side chain is conjugated to a substituent
HXEGSFTSELATILDXQAARDFIAWLKQHKITD

SEQ ID NO: 51 - protein, 33 aa, Artificial Sequence
  GLP-1/GLP-2 Dual agonist peptide
  MOD_RES (2)..(2): Aib
  MISC_FEATURE (16)..(16): Xaa is a residue of K, k (D-lys), R, Orn, Dap or Dab in which the side chain is conjugated to a substituent
HXEGSFTSELATILDXQAARDFIAWLIQQKITD

SEQ ID NO: 52 - protein, 33 aa, Artificial Sequence
  GLP-1/GLP-2 Dual agonist peptide
  MOD_RES (2)..(2): Aib
  MISC_FEATURE (16)..(16): Xaa is a residue of K, k (D-lys), R, Orn, Dap or Dab in which the side chain is conjugated to a substituent
HXEGSFTSELATILDXQAARDFIAWLIQYKITD

SEQ ID NO: 53 - protein, 33 aa, Artificial Sequence
  GLP-1/GLP-2 Dual agonist peptide
  MOD_RES (2)..(2): Aib
  MISC_FEATURE (16)..(16): Xaa is a residue of K, k (D-lys), R, Orn, Dap or Dab in which the side chain is conjugated to a substituent
HXEGTFSSELSTILEXQASREFIAWLIAYKITE

SEQ ID NO: 54 - protein, 39 aa, Artificial Sequence
  GLP-1/GLP-2 Dual agonist peptide
  MOD_RES (2)..(2): Aib
  MISC_FEATURE (34)..(38): Xaa at positions 34-38 is D-Lys
  MISC_FEATURE (39)..(39): Xaa is a residue of K, k (D-lys), R, Orn, Dap or Dab in which the side chain is conjugated to a substituent
HXEGTFSSELATILDEQAARDFIAWLIAHKITDXXXXXX

SEQ ID NO: 55 - protein, 39 aa, Artificial Sequence
  GLP-1/GLP-2 Dual agonist peptide
  MOD_RES (2)..(2): Aib
  MISC_FEATURE (34)..(38): Xaa at positions 34-38 is D-Lys
  MISC_FEATURE (39)..(39): Xaa is a residue of K, k (D-lys), R, Orn, Dap or Dab in which the side chain is conjugated to a substituent
HXEGTFTSELATILDEQAARDFIAWLIAHKITDXXXXXX

SEQ ID NO: 56 - protein, 39 aa, Artificial Sequence
  GLP-1/GLP-2 Dual agonist peptide
  MOD_RES (2)..(2): Aib
  MISC_FEATURE (34)..(38): Xaa at positions 34-38 is D-Lys
  MISC_FEATURE (39)..(39): Xaa is a residue of K, k (D-lys), R, Orn, Dap or Dab in which the side chain is conjugated to a substituent
HXEGSFTSELATILDEQAARDFIAWLIEHKITDXXXXXX

SEQ ID NO: 57 - protein, 33 aa, Artificial Sequence
  GLP-1/GLP-2 Dual agonist peptide
  MOD_RES (2)..(2): Aib
  MISC_FEATURE (10)..(10): Xaa is a residue of K, k (D-lys), R, Orn, Dap or Dab in which the side chain is conjugated to a substituent
HXEGSFTSEXATILDEQAARDFIAWLIEHKITD

SEQ ID NO: 58 - protein, 33 aa, Artificial Sequence
  GLP-1/GLP-2 Dual agonist peptide
  MOD_RES (2)..(2): Aib
  MISC_FEATURE (17)..(17): Xaa is a residue of K, k (D-lys), R, Orn, Dap or Dab in which the side chain is conjugated to a substituent
HXEGSFTSELATILEGXAARDFIAWLIEHKITD

SEQ ID NO: 59 - protein, 33 aa, Artificial Sequence
  GLP-1/GLP-2 Dual agonist peptide
  MOD_RES (2)..(2): Aib
  MISC_FEATURE (20)..(20): Xaa is a residue of K, k (D-lys), R, Orn, Dap or Dab in which the side chain is conjugated to a substituent
HXEGSFTSELATILDEQAAXDFIAWLIEHKITD

SEQ ID NO: 60 - protein, 33 aa, Artificial Sequence
  GLP-1/GLP-2 Dual agonist peptide
  MOD_RES (2)..(2): Aib
  MISC_FEATURE (20)..(20): Xaa is a residue of K, k (D-lys), R, Orn, Dap or Dab in which the side chain is conjugated to a substituent
HXEGTFTSELATILDEQAAXDFIAWLIEHKITD

SEQ ID NO: 61 - protein, 33 aa, Artificial Sequence
  GLP-1/GLP-2 Dual agonist peptide
  MOD_RES (2)..(2): Aib
  MISC_FEATURE (10)..(10): Xaa is a residue of K, k (D-lys), R, Orn, Dap or Dab in which the side chain is conjugated to a substituent
HXEGTFTSEXATILDEQAARDFIAWLIEHKITD

SEQ ID NO: 62 - protein, 33 aa, Artificial Sequence
  GLP-1/GLP-2 Dual agonist peptide
  MOD_RES (2)..(2): Aib
  MISC_FEATURE (17)..(17): Xaa is a residue of K, k (D-lys), R, Orn, Dap or Dab in which the side chain is conjugated to a substituent
HXEGSFTSELATILDAXAARDFIAWLIEHKITD

SEQ ID NO: 63 - protein, 33 aa, Artificial Sequence
  GLP-1/GLP-2 Dual agonist peptide
  MOD_RES (2)..(2): Aib
  MISC_FEATURE (20)..(20): Xaa is a residue of K, k (D-lys), R, Orn, Dap or Dab in which the side chain is conjugated to a substituent
HXEGSFTSELATILDAKAAXDFIAWLIEHKITD

SEQ ID NO: 64 - protein, 33 aa, Artificial Sequence; identical to SEQ ID NO: 17
  GLP-1/GLP-2 Dual agonist peptide
  MOD_RES (2)..(2): Aib
  MISC_FEATURE (16)..(16): Xaa indicates an L-lysine residue in which the side chain is conjugated to the substituent Z1- or Z1Z2

SEQ ID NO: 65 - protein, 33 aa, Artificial Sequence; identical to SEQ ID NO: 18
  GLP-1/GLP-2 Dual agonist peptide
  MOD_RES (2)..(2): Aib
  MISC_FEATURE (16)..(16): Xaa indicates an L-lysine residue in which the side chain is conjugated to the substituent Z1- or Z1Z2

SEQ ID NO: 66 - protein, 33 aa, Artificial Sequence; identical to SEQ ID NO: 19
  GLP-1/GLP-2 Dual agonist peptide
  MOD_RES (2)..(2): Aib
  MISC_FEATURE (16)..(16): Xaa indicates an L-lysine residue in which the side chain is conjugated to the substituent Z1- or Z1Z2

SEQ ID NO: 67 - protein, 33 aa, Artificial Sequence; identical to SEQ ID NO: 20
  GLP-1/GLP-2 Dual agonist peptide
  MOD_RES (2)..(2): Aib
  MISC_FEATURE (16)..(16): Xaa indicates an L-lysine residue in which the side chain is conjugated to the substituent Z1- or Z1Z2

SEQ ID NO: 68 - protein, 33 aa, Artificial Sequence; identical to SEQ ID NO: 21
  GLP-1/GLP-2 Dual agonist peptide
  MOD_RES (2)..(2): Aib
  MISC_FEATURE (16)..(16): Xaa indicates an L-lysine residue in which the side chain is conjugated to the substituent Z1- or Z1Z2

SEQ ID NO: 69 - protein, 33 aa, Artificial Sequence; identical to SEQ ID NO: 22
  GLP-1/GLP-2 Dual agonist peptide
  MOD_RES (2)..(2): Aib
  MISC_FEATURE (16)..(16): Xaa indicates an L-lysine residue in which the side chain is conjugated to the substituent Z1- or Z1Z2

SEQ ID NO: 70 - protein, 33 aa, Artificial Sequence; identical to SEQ ID NO: 23
  GLP-1/GLP-2 Dual agonist peptide
  MOD_RES (2)..(2): Aib
  MISC_FEATURE (17)..(17): Xaa indicates an L-lysine residue in which the side chain is conjugated to the substituent Z1- or Z1Z2

SEQ ID NO: 71 - protein, 33 aa, Artificial Sequence; identical to SEQ ID NO: 24
  GLP-1/GLP-2 Dual agonist peptide
  MOD_RES (2)..(2): Aib
  MISC_FEATURE (17)..(17): Xaa indicates an L-lysine residue in which the side chain is conjugated to the substituent Z1- or Z1Z2

SEQ ID NO: 72 - protein, 33 aa, Artificial Sequence; identical to SEQ ID NO: 25
  GLP-1/GLP-2 Dual agonist peptide
  MOD_RES (2)..(2): Aib
  MISC_FEATURE (17)..(17): Xaa indicates an L-lysine residue in which the side chain is conjugated to the substituent Z1- or Z1Z2

SEQ ID NO: 73 - protein, 33 aa, Artificial Sequence; identical to SEQ ID NO: 26
  GLP-1/GLP-2 Dual agonist peptide
  MOD_RES (2)..(2): Aib
  MISC_FEATURE (16)..(16): Xaa indicates an L-lysine residue in which the side chain is conjugated to the substituent Z1- or Z1Z2

SEQ ID NO: 74 - protein, 33 aa, Artificial Sequence; identical to SEQ ID NO: 27
  GLP-1/GLP-2 Dual agonist peptide
  MOD_RES (2)..(2): Aib
  MISC_FEATURE (16)..(16): Xaa indicates an L-lysine residue in which the side chain is conjugated to the substituent Z1- or Z1Z2

SEQ ID NO: 75 - protein, 33 aa, Artificial Sequence; identical to SEQ ID NO: 28
  GLP-1/GLP-2 Dual agonist peptide
  MOD_RES (2)..(2): Aib
  MISC_FEATURE (16)..(16): Xaa indicates an L-lysine residue in which the side chain is conjugated to the substituent Z1- or Z1Z2

SEQ ID NO: 76 - protein, 33 aa, Artificial Sequence; identical to SEQ ID NO: 29
  GLP-1/GLP-2 Dual agonist peptide
  MOD_RES (2)..(2): Aib
  MISC_FEATURE (16)..(16): Xaa indicates an L-lysine residue in which the side chain is conjugated to the substituent Z1- or Z1Z2

SEQ ID NO: 77 - protein, 33 aa, Artificial Sequence; identical to SEQ ID NO: 30
  GLP-1/GLP-2 Dual agonist peptide
  MOD_RES (2)..(2): Aib
  MISC_FEATURE (16)..(16): Xaa indicates an L-lysine residue in which the side chain is conjugated to the substituent Z1- or Z1Z2

SEQ ID NO: 78 - protein, 33 aa, Artificial Sequence; identical to SEQ ID NO: 31
  GLP-1/GLP-2 Dual agonist peptide
  MOD_RES (2)..(2): Aib
  MISC_FEATURE (16)..(16): Xaa indicates an L-lysine residue in which the side chain is conjugated to the substituent Z1- or Z1Z2

SEQ ID NO: 79 - protein, 33 aa, Artificial Sequence; identical to SEQ ID NO: 32
  GLP-1/GLP-2 Dual agonist peptide
  MOD_RES (2)..(2): Aib
  MISC_FEATURE (16)..(16): Xaa indicates an L-lysine residue in which the side chain is conjugated to the substituent Z1- or Z1Z2

SEQ ID NO: 80 - protein, 33 aa, Artificial Sequence; identical to SEQ ID NO: 33
  GLP-1/GLP-2 Dual agonist peptide
  MOD_RES (2)..(2): Aib
  MISC_FEATURE (16)..(16): Xaa indicates an L-lysine residue in which the side chain is conjugated to the substituent Z1- or Z1Z2

SEQ ID NO: 81 - protein, 33 aa, Artificial Sequence; identical to SEQ ID NO: 34
  GLP-1/GLP-2 Dual agonist peptide
  MOD_RES (2)..(2): Aib
  MISC_FEATURE (16)..(16): Xaa indicates an L-lysine residue in which the side chain is conjugated to the substituent Z1- or Z1Z2

SEQ ID NO: 82 - protein, 33 aa, Artificial Sequence; identical to SEQ ID NO: 35
  GLP-1/GLP-2 Dual agonist peptide
  MOD_RES (2)..(2): Aib
  MISC_FEATURE (16)..(16): Xaa indicates an L-lysine residue in which the side chain is conjugated to the substituent Z1- or Z1Z2

SEQ ID NO: 83 - protein, 33 aa, Artificial Sequence; identical to SEQ ID NO: 36
  GLP-1/GLP-2 Dual agonist peptide
  MOD_RES (2)..(2): Aib
  MISC_FEATURE (16)..(16): Xaa indicates an L-lysine residue in which the side chain is conjugated to the substituent Z1- or Z1Z2

SEQ ID NO: 84 - protein, 33 aa, Artificial Sequence; identical to SEQ ID NO: 37
  GLP-1/GLP-2 Dual agonist peptide
  MOD_RES (2)..(2): Aib
  MISC_FEATURE (16)..(16): Xaa indicates an L-lysine residue in which the side chain is conjugated to the substituent Z1- or Z1Z2

SEQ ID NO: 85 - protein, 33 aa, Artificial Sequence; identical to SEQ ID NO: 38
  GLP-1/GLP-2 Dual agonist peptide
  MOD_RES (2)..(2): Aib
  MISC_FEATURE (16)..(16): Xaa indicates an L-lysine residue respectively in which the side chain is conjugated to the substituent Z1- or Z1Z2

SEQ ID NO: 86 - protein, 33 aa, Artificial Sequence; identical to SEQ ID NO: 39
  GLP-1/GLP-2 Dual agonist peptide
  MOD_RES (2)..(2): Aib
  MISC_FEATURE (16)..(16): Xaa indicates an L-lysine residue in which the side chain is conjugated to the substituent Z1- or Z1Z2

SEQ ID NO: 87 - protein, 33 aa, Artificial Sequence; identical to SEQ ID NO: 40
  GLP-1/GLP-2 Dual agonist peptide
  MOD_RES (2)..(2): Aib
  MISC_FEATURE (16)..(16): Xaa indicates an L-lysine residue in which the side chain is conjugated to the substituent Z1- or Z1Z2

SEQ ID NO: 88 - protein, 33 aa, Artificial Sequence; identical to SEQ ID NO: 41
  GLP-1/GLP-2 Dual agonist peptide
  MOD_RES (2)..(2): Aib
  MISC_FEATURE (16)..(16): Xaa indicates an L-lysine residue in which the side chain is conjugated to the substituent Z1- or Z1Z2

SEQ ID NO: 89 - protein, 33 aa, Artificial Sequence; identical to SEQ ID NO: 42
  GLP-1/GLP-2 Dual agonist peptide
  MOD_RES (2)..(2): Aib
  MISC_FEATURE (16)..(16): Xaa indicates an L-lysine residue in which the side chain is conjugated to the substituent Z1- or Z1Z2

SEQ ID NO: 90 - protein, 33 aa, Artificial Sequence; identical to SEQ ID NO: 43
  GLP-1/GLP-2 Dual agonist peptide
  MOD_RES (2)..(2): Aib
  MISC_FEATURE (16)..(16): Xaa indicates an L-lysine residue in which the side chain is conjugated to the substituent Z1- or Z1Z2

SEQ ID NO: 91 - protein, 33 aa, Artificial Sequence; identical to SEQ ID NO: 44
  GLP-1/GLP-2 Dual agonist peptide
  MOD_RES (2)..(2): Aib
  MISC_FEATURE (16)..(16): Xaa indicates an L-lysine residue in which the side chain is conjugated to the substituent Z1- or Z1Z2

SEQ ID NO: 92 - protein, 33 aa, Artificial Sequence; identical to SEQ ID NO: 45
  GLP-1/GLP-2 Dual agonist peptide
  MOD_RES (2)..(2): Aib
  MISC_FEATURE (16)..(16): Xaa indicates an L-lysine residue in which the side chain is conjugated to the substituent Z1- or Z1Z2

SEQ ID NO: 93 - protein, 33 aa, Artificial Sequence; identical to SEQ ID NO: 46
  GLP-1/GLP-2 Dual agonist peptide
  MOD_RES (2)..(2): Aib
  MISC_FEATURE (16)..(16): Xaa indicates an L-lysine residue in which the side chain is conjugated to the substituent Z1- or Z1Z2

SEQ ID NO: 94 - protein, 33 aa, Artificial Sequence; identical to SEQ ID NO: 47
  GLP-1/GLP-2 Dual agonist peptide
  MOD_RES (2)..(2): Aib
  MISC_FEATURE (16)..(16): Xaa indicates an L-lysine residue in which the side chain is conjugated to the substituent Z1- or Z1Z2

SEQ ID NO: 95 - protein, 33 aa, Artificial Sequence; identical to SEQ ID NO: 48
  GLP-1/GLP-2 Dual agonist peptide
  MOD_RES (2)..(2): Aib
  MISC_FEATURE (16)..(16): Xaa indicates an L-lysine residue in which the side chain is conjugated to the substituent Z1- or Z1Z2

SEQ ID NO: 96 - protein, 33 aa, Artificial Sequence; identical to SEQ ID NO: 49
  GLP-1/GLP-2 Dual agonist peptide
  MOD_RES (2)..(2): Aib
  MISC_FEATURE (16)..(16): Xaa indicates an L-lysine residue in which the side chain is conjugated to the substituent Z1- or Z1Z2

SEQ ID NO: 97 - protein, 33 aa, Artificial Sequence; identical to SEQ ID NO: 50
  GLP-1/GLP-2 Dual agonist peptide
  MOD_RES (2)..(2): Aib
  MISC_FEATURE (16)..(16): Xaa indicates an L-lysine residue in which the side chain is conjugated to the substituent Z1- or Z1Z2

SEQ ID NO: 98 - protein, 33 aa, Artificial Sequence; identical to SEQ ID NO: 51
  GLP-1/GLP-2 Dual agonist peptide
  MOD_RES (2)..(2): Aib
  MISC_FEATURE (16)..(16): Xaa indicates an L-lysine residue in which the side chain is conjugated to the substituent Z1- or Z1Z2

SEQ ID NO: 99 - protein, 33 aa, Artificial Sequence; identical to SEQ ID NO: 52
  GLP-1/GLP-2 Dual agonist peptide
  MOD_RES (2)..(2): Aib
  MISC_FEATURE (16)..(16): Xaa indicates an L-lysine residue in which the side chain is conjugated to the substituent Z1- or Z1Z2

SEQ ID NO: 100 - protein, 33 aa, Artificial Sequence; identical to SEQ ID NO: 53
  GLP-1/GLP-2 Dual agonist peptide
  MOD_RES (2)..(2): Aib
  MISC_FEATURE (16)..(16): Xaa indicates an L-lysine residue in which the side chain is conjugated to the substituent Z1- or Z1Z2

SEQ ID NO: 101 - protein, 39 aa, Artificial Sequence; identical to SEQ ID NO: 54
  GLP-1/GLP-2 Dual agonist peptide
  MOD_RES (2)..(2): Aib
  MISC_FEATURE (34)..(38): Xaa at positions 34-38 is D-Lys
  MISC_FEATURE (39)..(39): Xaa indicates a D-lysine residue in which the side chain is conjugated to the substituent Z1- or Z1Z2

SEQ ID NO: 102 - protein, 39 aa, Artificial Sequence; identical to SEQ ID NO: 55
  GLP-1/GLP-2 Dual agonist peptide
  MOD_RES (2)..(2): Aib
  MISC_FEATURE (34)..(38): Xaa at positions 34-38 is D-Lys
  MISC_FEATURE (39)..(39): Xaa indicates a D-lysine residue in which the side chain is conjugated to the substituent Z1- or Z1Z2

SEQ ID NO: 103 - protein, 39 aa, Artificial Sequence; identical to SEQ ID NO: 56
  GLP-1/GLP-2 Dual agonist peptide
  MOD_RES (2)..(2): Aib
  MISC_FEATURE (34)..(38): Xaa at positions 34-38 is D-Lys
  MISC_FEATURE (39)..(39): Xaa indicates a D-lysine residue in which the side chain is conjugated to the substituent Z1- or Z1Z2

SEQ ID NO: 104 - protein, 33 aa, Artificial Sequence; identical to SEQ ID NO: 57
  GLP-1/GLP-2 Dual agonist peptide
  MOD_RES (2)..(2): Aib
  MISC_FEATURE (10)..(10): Xaa indicates an L-lysine residue in which the side chain is conjugated to the substituent Z1- or Z1Z2

SEQ ID NO: 105 - protein, 33 aa, Artificial Sequence; identical to SEQ ID NO: 58
  GLP-1/GLP-2 Dual agonist peptide
  MOD_RES (2)..(2): Aib
  MISC_FEATURE (17)..(17): Xaa indicates an L-lysine residue in which the side chain is conjugated to the substituent Z1- or Z1Z2

SEQ ID NO: 106 - protein, 33 aa, Artificial Sequence; identical to SEQ ID NO: 59
  GLP-1/GLP-2 Dual agonist peptide
  MOD_RES (2)..(2): Aib
  MISC_FEATURE (20)..(20): Xaa indicates an L-lysine residue in which the side chain is conjugated to the substituent Z1- or Z1Z2

SEQ ID NO: 107 - protein, 33 aa, Artificial Sequence; identical to SEQ ID NO: 60
  GLP-1/GLP-2 Dual agonist peptide
  MOD_RES (2)..(2): Aib
  MISC_FEATURE (20)..(20): Xaa indicates an L-lysine residue in which the side chain is conjugated to the substituent Z1- or Z1Z2

SEQ ID NO: 108 - protein, 33 aa, Artificial Sequence; identical to SEQ ID NO: 61
  GLP-1/GLP-2 Dual agonist peptide
  MOD_RES (2)..(2): Aib
  MISC_FEATURE (10)..(10): Xaa indicates an L-lysine residue in which the side chain is conjugated to the substituent Z1- or Z1Z2

SEQ ID NO: 109 - protein, 33 aa, Artificial Sequence; identical to SEQ ID NO: 62
  GLP-1/GLP-2 Dual agonist peptide
  MOD_RES (2)..(2): Aib
  MISC_FEATURE (17)..(17): Xaa indicates an L-lysine residue in which the side chain is conjugated to the substituent Z1- or Z1Z2

SEQ ID NO: 110 - protein, 33 aa, Artificial Sequence; identical to SEQ ID NO: 63
  GLP-1/GLP-2 Dual agonist peptide
  MOD_RES (2)..(2): Aib
  MISC_FEATURE (20)..(20): Xaa indicates an L-lysine residue in which the side chain is conjugated to the substituent Z1- or Z1Z2

SEQ ID NO: 111 - protein, 33 aa, Artificial Sequence; identical to SEQ ID NO: 17
  GLP-1/GLP-2 Dual agonist peptide
  MOD_RES (2)..(2): Aib
  MISC_FEATURE (16)..(16): Xaa is K([17-carboxy-heptadecanoyl]-isoGlu)

SEQ ID NO: 112 - protein, 33 aa, Artificial Sequence; identical to SEQ ID NO: 18
  GLP-1/GLP-2 Dual agonist peptide
  MOD_RES (2)..(2): Aib
  MISC_FEATURE (16)..(16): Xaa is K([17-carboxy-heptadecanoyl]-isoGlu)

SEQ ID NO: 113 - protein, 33 aa, Artificial Sequence; identical to SEQ ID NO: 19
  GLP-1/GLP-2 Dual agonist peptide
  MOD_RES (2)..(2): Aib
  MISC_FEATURE (16)..(16): Xaa is K([17-carboxy-heptadecanoyl]-isoGlu)

SEQ ID NO: 114 - protein, 33 aa, Artificial Sequence; identical to SEQ ID NO: 20
  GLP-1/GLP-2 Dual agonist peptide
  MOD_RES (2)..(2): Aib
  MISC_FEATURE (16)..(16): Xaa is K([17-carboxy-heptadecanoyl]-isoGlu)

SEQ ID NO: 115 - protein, 33 aa, Artificial Sequence; identical to SEQ ID NO: 21
  GLP-1/GLP-2 Dual agonist peptide
  MOD_RES (2)..(2): Aib
  MISC_FEATURE (16)..(16): Xaa is K([17-carboxy-heptadecanoyl]-isoGlu)

SEQ ID NO: 116 - protein, 33 aa, Artificial Sequence; identical to SEQ ID NO: 22
  GLP-1/GLP-2 Dual agonist peptide
  MOD_RES (2)..(2): Aib
  MISC_FEATURE (16)..(16): Xaa is K([17-carboxy-heptadecanoyl]-isoGlu)

SEQ ID NO: 117 - protein, 33 aa, Artificial Sequence; identical to SEQ ID NO: 23
  GLP-1/GLP-2 Dual agonist peptide
  MOD_RES (2)..(2): Aib
  MISC_FEATURE (17)..(17): Xaa is K([17-carboxy-heptadecanoyl]-isoGlu)

SEQ ID NO: 118 - protein, 33 aa, Artificial Sequence; identical to SEQ ID NO: 24
  GLP-1/GLP-2 Dual agonist peptide
  MOD_RES (2)..(2): Aib
  MISC_FEATURE (17)..(17): Xaa is K([17-carboxy-heptadecanoyl]-isoGlu)

SEQ ID NO: 119 - protein, 33 aa, Artificial Sequence; identical to SEQ ID NO: 25
  GLP-1/GLP-2 Dual agonist peptide
  MOD_RES (2)..(2): Aib
  MISC_FEATURE (17)..(17): Xaa  is K([17-carboxy-heptadecanoyl]-isoGlu)

SEQ ID NO: 120 - protein, 33 aa, Artificial Sequence; identical to SEQ ID NO: 26
  GLP-1/GLP-2 Dual agonist peptide
  MOD_RES (2)..(2): Aib
  MISC_FEATURE (16)..(16): Xaa is K([17-carboxy-heptadecanoyl]-isoGlu)

SEQ ID NO: 121 - protein, 33 aa, Artificial Sequence; identical to SEQ ID NO: 27
  GLP-1/GLP-2 Dual agonist peptide
  MOD_RES (2)..(2): Aib
  MISC_FEATURE (16)..(16): Xaa is K([17-carboxy-heptadecanoyl]-isoGlu)

SEQ ID NO: 122 - protein, 33 aa, Artificial Sequence; identical to SEQ ID NO: 28
  GLP-1/GLP-2 Dual agonist peptide
  MOD_RES (2)..(2): Aib
  MISC_FEATURE (16)..(16): Xaa is K([17-carboxy-heptadecanoyl]-isoGlu)

SEQ ID NO: 123 - protein, 33 aa, Artificial Sequence; identical to SEQ ID NO: 29
  GLP-1/GLP-2 Dual agonist peptide
  MOD_RES (2)..(2): Aib
  MISC_FEATURE (16)..(16): Xaa is K([17-carboxy-heptadecanoyl]-isoGlu)

SEQ ID NO: 124 - protein, 33 aa, Artificial Sequence; identical to SEQ ID NO: 30
  GLP-1/GLP-2 Dual agonist peptide
  MOD_RES (2)..(2): Aib
  MISC_FEATURE (16)..(16): Xaa is K([17-carboxy-heptadecanoyl]-isoGlu)

SEQ ID NO: 125 - protein, 33 aa, Artificial Sequence; identical to SEQ ID NO: 31
  GLP-1/GLP-2 Dual agonist peptide
  MOD_RES (2)..(2): Aib
  MISC_FEATURE (16)..(16): Xaa is K([17-carboxy-heptadecanoyl]-isoGlu)

SEQ ID NO: 126 - protein, 33 aa, Artificial Sequence; identical to SEQ ID NO: 32
  GLP-1/GLP-2 Dual agonist peptide
  MOD_RES (2)..(2): Aib
  MISC_FEATURE (16)..(16): Xaa is K([17-carboxy-heptadecanoyl]-isoGlu)

SEQ ID NO: 127 - protein, 33 aa, Artificial Sequence; identical to SEQ ID NO: 33
  GLP-1/GLP-2 Dual agonist peptide
  MOD_RES (2)..(2): Aib
  MISC_FEATURE (16)..(16): Xaa is K([17-carboxy-heptadecanoyl]-isoGlu)

SEQ ID NO: 128 - protein, 33 aa, Artificial Sequence; identical to SEQ ID NO: 34
  GLP-1/GLP-2 Dual agonist peptide
  MOD_RES (2)..(2): Aib
  MISC_FEATURE (16)..(16): Xaa is K([17-carboxy-heptadecanoyl]-isoGlu)

SEQ ID NO: 129 - protein, 33 aa, Artificial Sequence; identical to SEQ ID NO: 35
  GLP-1/GLP-2 Dual agonist peptide
  MOD_RES (2)..(2): Aib
  MISC_FEATURE (16)..(16): Xaa is K([17-carboxy-heptadecanoyl]-isoGlu)

SEQ ID NO: 130 - protein, 33 aa, Artificial Sequence; identical to SEQ ID NO: 36
  GLP-1/GLP-2 Dual agonist peptide
  MOD_RES (2)..(2): Aib
  MISC_FEATURE (16)..(16): Xaa is K([17-carboxy-heptadecanoyl]-isoGlu)

SEQ ID NO: 131 - protein, 33 aa, Artificial Sequence; identical to SEQ ID NO: 37
  GLP-1/GLP-2 Dual agonist peptide
  MOD_RES (2)..(2): Aib
  MISC_FEATURE (16)..(16): Xaa is K([17-carboxy-heptadecanoyl]-isoGlu)

SEQ ID NO: 132 - protein, 33 aa, Artificial Sequence; identical to SEQ ID NO: 38
  GLP-1/GLP-2 Dual agonist peptide
  MOD_RES (2)..(2): Aib
  MISC_FEATURE (16)..(16): Xaa is K([17-carboxy-heptadecanoyl]-isoGlu)

SEQ ID NO: 133 - protein, 33 aa, Artificial Sequence; identical to SEQ ID NO: 39
  GLP-1/GLP-2 Dual agonist peptide
  MOD_RES (2)..(2): Aib
  MISC_FEATURE (16)..(16): Xaa is K([17-carboxy-heptadecanoyl]-isoGlu)

SEQ ID NO: 134 - protein, 33 aa, Artificial Sequence; identical to SEQ ID NO: 40
  GLP-1/GLP-2 Dual agonist peptide
  MOD_RES (2)..(2): Aib
  MISC_FEATURE (16)..(16): Xaa is K([17-carboxy-heptadecanoyl]-isoGlu)

SEQ ID NO: 135 - protein, 33 aa, Artificial Sequence; identical to SEQ ID NO: 41
  GLP-1/GLP-2 Dual agonist peptide
  MOD_RES (2)..(2): Aib
  MISC_FEATURE (16)..(16): Xaa is K([17-carboxy-heptadecanoyl]-isoGlu)

SEQ ID NO: 136 - protein, 33 aa, Artificial Sequence; identical to SEQ ID NO: 42
  GLP-1/GLP-2 Dual agonist peptide
  MOD_RES (2)..(2): Aib
  MISC_FEATURE (16)..(16): Xaa is K([17-carboxy-heptadecanoyl]-isoGlu)

SEQ ID NO: 137 - protein, 33 aa, Artificial Sequence; identical to SEQ ID NO: 43
  GLP-1/GLP-2 Dual agonist peptide
  MOD_RES (2)..(2): Aib
  MISC_FEATURE (16)..(16): Xaa is K([17-carboxy-heptadecanoyl]-isoGlu)

SEQ ID NO: 138 - protein, 33 aa, Artificial Sequence; identical to SEQ ID NO: 44
  GLP-1/GLP-2 Dual agonist peptide
  MOD_RES (2)..(2): Aib
  MISC_FEATURE (16)..(16): Xaa is K([17-carboxy-heptadecanoyl]-isoGlu)

SEQ ID NO: 139 - protein, 33 aa, Artificial Sequence; identical to SEQ ID NO: 45
  GLP-1/GLP-2 Dual agonist peptide
  MOD_RES (2)..(2): Aib
  MISC_FEATURE (16)..(16): Xaa is K([17-carboxy-heptadecanoyl]-isoGlu)

SEQ ID NO: 140 - protein, 33 aa, Artificial Sequence; identical to SEQ ID NO: 46
  GLP-1/GLP-2 Dual agonist peptide
  MOD_RES (2)..(2): Aib
  MISC_FEATURE (16)..(16): Xaa is K([17-carboxy-heptadecanoyl]-isoGlu)

SEQ ID NO: 141 - protein, 33 aa, Artificial Sequence; identical to SEQ ID NO: 47
  GLP-1/GLP-2 Dual agonist peptide
  MOD_RES (2)..(2): Aib
  misc (16)..(16): Xaa is K([17-carboxy-heptadecanoyl]-isoGlu)

SEQ ID NO: 142 - protein, 33 aa, Artificial Sequence; identical to SEQ ID NO: 48
  GLP-1/GLP-2 Dual agonist peptide
  MOD_RES (2)..(2): Aib
  MISC_FEATURE (16)..(16): Xaa is K([Hexadecanoyl]-betaAla)

SEQ ID NO: 143 - protein, 33 aa, Artificial Sequence; identical to SEQ ID NO: 49
  GLP-1/GLP-2 Dual agonist peptide
  MOD_RES (2)..(2): Aib
  MISC_FEATURE (16)..(16): Xaa is K([17-carboxy-heptadecanoyl]iso-Glu-Peg3)

SEQ ID NO: 144 - protein, 33 aa, Artificial Sequence; identical to SEQ ID NO: 50
  GLP-1/GLP-2 Dual agonist peptide
  MOD_RES (2)..(2): Aib
  MISC_FEATURE (16)..(16): Xaa is K([19-carboxy-nonadecanoyl]iso-Glu-Peg3-Peg3)

SEQ ID NO: 145 - protein, 33 aa, Artificial Sequence; identical to SEQ ID NO: 51
  GLP-1/GLP-2 Dual agonist peptide
  MOD_RES (2)..(2): Aib
  MISC_FEATURE (16)..(16): Xaa is K([19-carboxy-nonadecanoyl]iso-Lys-Peg3-Peg3-Peg3)

SEQ ID NO: 146 - protein, 33 aa, Artificial Sequence; identical to SEQ ID NO: 52
  GLP-1/GLP-2 Dual agonist peptide
  MOD_RES (2)..(2): Aib
  MISC_FEATURE (16)..(16): Xaa is K(Octadecanoyl)

SEQ ID NO: 147 - protein, 33 aa, Artificial Sequence; identical to SEQ ID NO: 53
  GLP-1/GLP-2 Dual agonist peptide
  MOD_RES (2)..(2): Aib
  MISC_FEATURE (16)..(16): Xaa is K(Hexadecanoyl-isoGlu)

SEQ ID NO: 148 - protein, 39 aa, Artificial Sequence; identical to SEQ ID NO: 54
  GLP-1/GLP-2 Dual agonist peptide
  MOD_RES (2)..(2): Aib
  MISC_FEATURE (34)..(38): Xaa at positions 34-38 is D-Lys
  MISC_FEATURE (39)..(39): Xaa is a D-lysine residue in which the side chain is conjugated to ([17-carboxy-Heptadecanoyl]-isoGlu)

SEQ ID NO: 149 - protein, 39 aa, Artificial Sequence; identical to SEQ ID NO: 55
  GLP-1/GLP-2 Dual agonist peptide
  MOD_RES (2)..(2): Aib
  MISC_FEATURE (34)..(38): Xaa at positions 34-38 is D-Lys
  MISC_FEATURE (39)..(39): Xaa is a D-lysine residue in which the side chain is conjugated to ([17-carboxy-Heptadecanoyl]-isoGlu)

SEQ ID NO: 150 - protein, 39 aa, Artificial Sequence; identical to SEQ ID NO: 56
  GLP-1/GLP-2 Dual agonist peptide
  MOD_RES (2)..(2): Aib
  MISC_FEATURE (34)..(38): Xaa at positions 34-38 is D-Lys
  MISC_FEATURE (39)..(39): Xaa is a D-lysine residue in which the side chain is conjugated to ([17-carboxy-Heptadecanoyl]-isoGlu)

SEQ ID NO: 151 - protein, 33 aa, Artificial Sequence; identical to SEQ ID NO: 35
  GLP-1/GLP-2 Dual agonist peptide
  MOD_RES (2)..(2): Aib
  MISC_FEATURE (16)..(16): Xaa is K([19-Carboxy-nonadecanoyl]-isoGlu)

SEQ ID NO: 152 - protein, 33 aa, Artificial Sequence; identical to SEQ ID NO: 57
  GLP-1/GLP-2 Dual agonist peptide
  MOD_RES (2)..(2): Aib
  MISC_FEATURE (10)..(10): Xaa is K([19-carboxy-nonadecanoyl]iso-Glu-Peg3-Peg3)

SEQ ID NO: 153 - protein, 33 aa, Artificial Sequence; identical to SEQ ID NO: 21
  GLP-1/GLP-2 Dual agonist peptide
  MOD_RES (2)..(2): Aib
  MISC_FEATURE (16)..(16): Xaa is K([19-carboxy-nonadecanoyl]iso-Glu-Peg3-Peg3)

SEQ ID NO: 154 - protein, 33 aa, Artificial Sequence; identical to SEQ ID NO: 58
  GLP-1/GLP-2 Dual agonist peptide
  MOD_RES (2)..(2): Aib
  MISC_FEATURE (17)..(17): Xaa is K([19-carboxy-nonadecanoyl]iso-Glu-Peg3-Peg3)

SEQ ID NO: 155 - protein, 33 aa, Artificial Sequence; identical to SEQ ID NO: 59
  GLP-1/GLP-2 Dual agonist peptide
  MOD_RES (2)..(2): Aib
  MISC_FEATURE (20)..(20): Xaa is K([19-carboxy-nonadecanoyl]iso-Glu-Peg3-Peg3)

SEQ ID NO: 156 - protein, 33 aa, Artificial Sequence; identical to SEQ ID NO: 60
  GLP-1/GLP-2 Dual agonist peptide
  MOD_RES (2)..(2): Aib
  MISC_FEATURE (20)..(20): Xaa is K([19-carboxy-nonadecanoyl]iso-Glu-Peg3-Peg3)

SEQ ID NO: 157 - protein, 33 aa, Artificial Sequence; identical to SEQ ID NO: 33
  GLP-1/GLP-2 Dual agonist peptide
  MOD_RES (2)..(2): Aib
  MISC_FEATURE (16)..(16): Xaa is K([17-Carboxy-heptadecanoyl]-isoGlu-KEK-Peg3)

SEQ ID NO: 158 - protein, 33 aa, Artificial Sequence; identical to SEQ ID NO: 33
  GLP-1/GLP-2 Dual agonist peptide
  MOD_RES (2)..(2): Aib
  MISC_FEATURE (16)..(16): Xaa is K([19-Carboxy-nonadecanoyl]-isoGlu-KEK-Peg3)

SEQ ID NO: 159 - protein, 33 aa, Artificial Sequence; identical to SEQ ID NO: 36
  GLP-1/GLP-2 Dual agonist peptide
  MOD_RES (2)..(2): Aib
  MISC_FEATURE (16)..(16): Xaa is K([17-Carboxy-heptadecanoyl]-isoGlu-KEK-Peg3)

SEQ ID NO: 160 - protein, 33 aa, Artificial Sequence; identical to SEQ ID NO: 36
  GLP-1/GLP-2 Dual agonist peptide
  MOD_RES (2)..(2): Aib
  MISC_FEATURE (16)..(16): Xaa is K([19-Carboxy-nonadecanoyl]-isoGlu-KEK-Peg3)

SEQ ID NO: 161 - protein, 33 aa, Artificial Sequence; identical to SEQ ID NO: 35
  GLP-1/GLP-2 Dual agonist peptide
  MOD_RES (2)..(2): Aib
  MISC_FEATURE (16)..(16): Xaa is K([19-Carboxy-nonadecanoyl]-isoGlu-KEK)

SEQ ID NO: 162 - protein, 33 aa, Artificial Sequence; identical to SEQ ID NO: 35
  GLP-1/GLP-2 Dual agonist peptide
  MOD_RES (2)..(2): Aib
  MISC_FEATURE (16)..(16): Xaa is K([19-Carboxy-nonadecanoyl]-isoGlu-KEK-Peg3)

SEQ ID NO: 163 - protein, 33 aa, Artificial Sequence; identical to SEQ ID NO: 57
  GLP-1/GLP-2 Dual agonist peptide
  MOD_RES (2)..(2): Aib
  MISC_FEATURE (10)..(10): Xaa is K([19-Carboxy-nonadecanoyl]-isoGlu-KEK-Peg3)

SEQ ID NO: 164 - protein, 33 aa, Artificial Sequence; identical to SEQ ID NO: 61
  GLP-1/GLP-2 Dual agonist peptide
  MOD_RES (2)..(2): Aib
  MISC_FEATURE (10)..(10): Xaa is K([19-Carboxy-nonadecanoyl]-isoGlu-KEK-Peg3)

SEQ ID NO: 165 - protein, 33 aa, Artificial Sequence; identical to SEQ ID NO: 57
  GLP-1/GLP-2 Dual agonist peptide
  MOD_RES (2)..(2): Aib
  MISC_FEATURE (10)..(10): Xaa is K([19-carboxy-nonadecanoyl]iso-Glu-KEK-Peg3-Peg3)

SEQ ID NO: 166 - protein, 33 aa, Artificial Sequence; identical to SEQ ID NO: 41
  GLP-1/GLP-2 Dual agonist peptide
  MOD_RES (2)..(2): Aib
  MISC_FEATURE (16)..(16): Xaa is K([19-Carboxy-nonadecanoyl]-isoGlu-KEK-Peg3)

SEQ ID NO: 167 - protein, 33 aa, Artificial Sequence; identical to SEQ ID NO: 40
  GLP-1/GLP-2 Dual agonist peptide
  MOD_RES (2)..(2): Aib
  MISC_FEATURE (16)..(16): Xaa is K([19-Carboxy-nonadecanoyl]-isoGlu-KEK-Peg3)

SEQ ID NO: 168 - protein, 33 aa, Artificial Sequence; identical to SEQ ID NO: 38
  GLP-1/GLP-2 Dual agonist peptide
  MOD_RES (2)..(2): Aib
  MISC_FEATURE (16)..(16): Xaa is K([19-Carboxy-nonadecanoyl]-isoGlu-KEK-Peg3)

SEQ ID NO: 169 - protein, 33 aa, Artificial Sequence; identical to SEQ ID NO: 21
  GLP-1/GLP-2 Dual agonist peptide
  MOD_RES (2)..(2): Aib
  MISC_FEATURE (16)..(16): Xaa is K([19-Carboxy-nonadecanoyl]-isoGlu-KEK-Peg3)

SEQ ID NO: 170 - protein, 33 aa, Artificial Sequence; identical to SEQ ID NO: 40
  GLP-1/GLP-2 Dual agonist peptide
  MOD_RES (2)..(2): Aib
  MISC_FEATURE (16)..(16): Xaa is K([19-carboxy-nonadecanoyl]iso-Glu-KEK-Peg3-Peg3)

SEQ ID NO: 171 - protein, 33 aa, Artificial Sequence; identical to SEQ ID NO: 58
  GLP-1/GLP-2 Dual agonist peptide
  MOD_RES (2)..(2): Aib
  MISC_FEATURE (17)..(17): Xaa is K([19-Carboxy-nonadecanoyl]-isoGlu-KEK-Peg3)

SEQ ID NO: 172 - protein, 33 aa, Artificial Sequence; identical to SEQ ID NO: 62
  GLP-1/GLP-2 Dual agonist peptide
  MOD_RES (2)..(2): Aib
  MISC_FEATURE (17)..(17): Xaa is K([19-Carboxy-nonadecanoyl]-isoGlu-KEK-Peg3)

SEQ ID NO: 173 - protein, 33 aa, Artificial Sequence; identical to SEQ ID NO: 62
  GLP-1/GLP-2 Dual agonist peptide
  MOD_RES (2)..(2): Aib
  MISC_FEATURE (17)..(17): Xaa is K([19-carboxy-nonadecanoyl]iso-Glu-KEK-Peg3-Peg3)

SEQ ID NO: 174 - protein, 33 aa, Artificial Sequence; identical to SEQ ID NO: 59
  GLP-1/GLP-2 Dual agonist peptide
  MOD_RES (2)..(2): Aib
  MISC_FEATURE (20)..(20): Xaa is K([19-Carboxy-nonadecanoyl]-isoGlu-KEK-Peg3)

SEQ ID NO: 175 - protein, 33 aa, Artificial Sequence; identical to SEQ ID NO: 60
  GLP-1/GLP-2 Dual agonist peptide
  MOD_RES (2)..(2): Aib
  MISC_FEATURE (20)..(20): Xaa is K([19-Carboxy-nonadecanoyl]-isoGlu-KEK-Peg3)

SEQ ID NO: 176 - protein, 33 aa, Artificial Sequence; identical to SEQ ID NO: 59
  GLP-1/GLP-2 Dual agonist peptide
  MOD_RES (2)..(2): Aib
  MISC_FEATURE (20)..(20): Xaa is K([19-carboxy-nonadecanoyl]iso-Glu-KEK-Peg3-Peg3)

SEQ ID NO: 177 - protein, 33 aa, Artificial Sequence; identical to SEQ ID NO: 60
  GLP-1/GLP-2 Dual agonist peptide
  MOD_RES (2)..(2): Aib
  MISC_FEATURE (20)..(20): Xaa is K([19-carboxy-nonadecanoyl]iso-Glu-KEK-Peg3-Peg3)

SEQ ID NO: 178 - protein, 33 aa, Artificial Sequence; identical to SEQ ID NO: 63
  GLP-1/GLP-2 Dual agonist peptide
  MOD_RES (2)..(2): Aib
  MISC_FEATURE (20)..(20): Xaa is K([19-Carboxy-nonadecanoyl]-isoGlu-KEK-Peg3)